European Patent Application EP 4 467 155 A1, published November 27, 2024. Title: CAR-Thy Treg CELLS, COMPOSITIONS AND USES THEREOF IN IMMUNOTHERAPY. Applicant: Fundación para la investigación sanitaria Gregorio Marañón (FIBHGM). The sequence listing filed with the application follows.

SEQUENCE LISTING (12 sequences)

SEQ ID NO: 1 - protein, 42 aa, Homo sapiens
  source 1..42: note = 41-BB domain
KRGRKKLLYIFKQPFMRPVQTTQEEDGCSCRFPEEEEGGCEL

SEQ ID NO: 2 - protein, 142 aa, Streptomyces avidinii
  source 1..142: note = High affinity monomeric streptavidin domain
METDTLLLWVLLLWVPGSTGGAEAGITGTWYNQHGSTFTVTAGADGNLTGQYENRAQGTGCQNSPYTLTGRYNGTKLEWRVEWNNSTENCHSRTEWRGQYQGGAEARINTQWNLTYEGGSGPATEQGQDTFTKVKPSAASGS

SEQ ID NO: 3 - protein, 45 aa, Homo sapiens
  source 1..45: note = CD8a hinge
TTTPAPRPPTPAPTIASQPLSLRPEACRPAAGGAVHTRGLDFACD

SEQ ID NO: 4 - protein, 28 aa, Homo sapiens
  source 1..28: note = CD28 transmembrane domain
MFWVLVVVGGVLACYSLLVTVAFIIFWV

SEQ ID NO: 5 - protein, 112 aa, Homo sapiens
  source 1..112: note = CD3zeta
RVKFSRSADAPAYQQGQNQLYNELNLGRREEYDVLDKRRGRDPEMGGKPRRKNPQEGLYNELQKDKMAEAYSEIGMKGERRRGKGHDGLYQGLSTATKDTYDALHMQALPPR

SEQ ID NO: 6 - protein, 369 aa, synthetic construct
  source 1..369: note = Complete amino acid sequence of CAR41-BB
METDTLLLWVLLLWVPGSTGGAEAGITGTWYNQHGSTFTVTAGADGNLTGQYENRAQGTGCQNSPYTLTGRYNGTKLEWRVEWNNSTENCHSRTEWRGQYQGGAEARINTQWNLTYEGGSGPATEQGQDTFTKVKPSAASGSTTTPAPRPPTPAPTIASQPLSLRPEACRPAAGGAVHTRGLDFACDMFWVLVVVGGVLACYSLLVTVAFIIFWVKRGRKKLLYIFKQPFMRPVQTTQEEDGCSCRFPEEEEGGCELRVKFSRSADAPAYQQGQNQLYNELNLGRREEYDVLDKRRGRDPEMGGKPRRKNPQEGLYNELQKDKMAEAYSEIGMKGERRRGKGHDGLYQGLSTATKDTYDALHMQALPPR

SEQ ID NO: 7 - DNA, 1047 bp, synthetic construct
  source 1..1047: mol_type = other DNA; note = Sequence encoding for CAR41-BB
ggcgcagaggcgggtatcaccgggacatggtacaaccaacacggaagcacatttacagtcaccgctggagcagacgggaatctgaccggacagtacgagaacagggctcaggggacaggttgtcagaacagtccgtatactctgactgggaggtacaatggcacgaagctggagtggcgagtcgagtggaataattccacggaaaactgtcacagtagaacagagtggaggggacagtaccaggggggagcagaggcccggatcaacacccaatggaacttgacatatgaaggcgggtcaggccccgcgacagagcaaggacaggatacattcacgaaggtcaagccaagcgcagcctctggctctaccacaactccagctccccggccccctactcctgctccaaccattgcctcacagccactgagcctgcggcccgaagcttgtagacctgctgctggaggagctgtgcataccagaggcctggacttcgcctgcgatatgttctgggtgctggtggtggtgggcggggtgctggcctgctacagcctgctggtgacagtggccttcatcatcttttgggtgaaacggggcagaaagaaactcctgtatatattcaaacaaccatttatgagaccagtacaaactactcaagaggaagatggctgtagctgccgatttccagaagaagaagaaggaggatgtgaactgcgggtgaagttcagcagaagcgccgacgcccctgcctaccagcagggccagaatcagctgtacaacgagctgaacctgggcagaagggaagagtacgacgtcctggataagcggagaggccgggaccctgagatgggcggcaagcctcggcggaagaacccccaggaaggcctgtataacgaactgcagaaagacaagatggccgaggcctacagcgagatcggcatgaagggcgagcggaggcggggcaagggccacgacggcctgtatcagggcctgtccaccgccaccaaggatacctacgacgccctgcacatgcaggccctgcccccaagg

SEQ ID NO: 8 - DNA, 9517 bp, synthetic construct
  source 1..9517: mol_type = other DNA; note = Expression construct
tggaagggctaattcactcccaaagaagacaagatatccttgatctgtggatctaccacacacaaggctacttccctgattagcagaactacacaccagggccaggggtcagatatccactgacctttggatggtgctacaagctagtaccagttgagccagataaggtagaagaggccaataaaggagagaacaccagcttgttacaccctgtgagcctgcatgggatggatgacccggagagagaagtgttagagtggaggtttgacagccgcctagcatttcatcacgtggcccgagagctgcatccggagtacttcaagaactgctgatatcgagcttgctacaagggactttccgctggggactttccagggaggcgtggcctgggcgggactggggagtggcgagccctcagatcctgcatataagcagctgctttttgcctgtactgggtctctctggttagaccagatctgagcctgggagctctctggctaactagggaacccactgcttaagcctcaataaagcttgccttgagtgcttcaagtagtgtgtgcccgtctgttgtgtgactctggtaactagagatccctcagacccttttagtcagtgtggaaaatctctagcagtggcgcccgaacagggacttgaaagcgaaagggaaaccagaggagctctctcgacgcaggactcggcttgctgaagcgcgcacggcaagaggcgaggggcggcgactggtgagtacgccaaaaattttgactagcggaggctagaaggagagagatgggtgcgagagcgtcagtattaagcgggggagaattagatcgcgatgggaaaaaattcggttaaggccagggggaaagaaaaaatataaattaaaacatatagtatgggcaagcagggagctagaacgattcgcagttaatcctggcctgttagaaacatcagaaggctgtagacaaatactgggacagctacaaccatcccttcagacaggatcagaagaacttagatcattatataatacagtagcaaccctctattgtgtgcatcaaaggatagagataaaagacaccaaggaagctttagacaagatagaggaagagcaaaacaaaagtaagaccaccgcacagcaagcggccggccgctgatcttcagacctggaggaggagatatgagggacaattggagaagtgaattatataaatataaagtagtaaaaattgaaccattaggagtagcacccaccaaggcaaagagaagagtggtgcagagagaaaaaagagcagtgggaataggagctttgttccttgggttcttgggagcagcaggaagcactatgggcgcagcgtcaatgacgctgacggtacaggccagacaattattgtctggtatagtgcagcagcagaacaatttgctgagggctattgaggcgcaacagcatctgttgcaactcacagtctggggcatcaagcagctccaggcaagaatcctggctgtggaaagatacctaaaggatcaacagctcctggggatttggggttgctctggaaaactcatttgcaccactgctgtgccttggaatgctagttggagtaataaatctctggaacagatttggaatcacacgacctggatggagtgggacagagaaattaacaattacacaagcttaatacactccttaattgaagaatcgcaaaaccagcaagaaaagaatgaacaagaattattggaattagataaatgggcaagtttgtggaattggtttaacataacaaattggctgtggtatataaaattattcataatgatagtaggaggcttggtaggtttaagaatagtttttgctgtactttctatagtgaatagagttaggcagggatattcaccattatcgtttcagacccacctcccaaccccgaggggacccgacaggcccgaaggaatagaagaagaaggtggagagagagacagagacagatccattcgattagtgaacggatctcgacggtatcgcctttaaaagaaaaggggggattggggggtacagtgcaggggaaagaatagtagacataatagcaacagacatacaaactaaagaattacaaaaacaaattacaaaaattcaaaattttcgggtttattacagggacagcagagatccagtttatcgatgagtaattcatacaaaaggactcgcccctgccttggggaatcccagggaccgtcgttaaactcccactaacgtagaacccagagatcgctgcgttcccgccccctcacccgcccgctctcgtcatcactgaggtggagaagagcatgcgtgaggctccggtgcccgtcagtgggcagagcgcacatcgcccacagtccccgagaagttggggggaggggtcggcaattgaaccggtgcctagagaaggtggcgcggggtaaactgggaaagtgatgtcgtgtactggctccgcctttttcccgagggtgggggagaaccgtatataagtgcagtagtcgccgtgaacgttctttttcgcaacgggtttgccgccagaacacaggtaagtgccgtgtgtggttcccgcgggcctggcctctttacgggttatggcccttgcgtgccttgaattacttccacgcccctggctgcagtacgtgattcttgatcccgagcttcgggttggaagtgggtgggagagttcgaggccttgcgcttaaggagccccttcgcctcgtgcttgagttgaggcctggcttgggcgctggggccgccgcgtgcgaatctggtggcaccttcgcgcctgtctcgctgctttcgataagtctctagccatttaaaatttttgatgacctgctgcgacgctttttttctggcaagatagtcttgtaaatgcgggccaagatctgcacactggtatttcggtttttggggccgcgggcggcgacggggcccgtgcgtcccagcgcacatgttcggcgaggcggggcctgcgagcgcggccaccgagaatcggacgggggtagtctcaagctggccggcctgctctggtgcctggcctcgcgccgccgtgtatcgccccgccctgggcggcaaggctggcccggtcggcaccagttgcgtgagcggaaagatggccgcttcccggccctgctgcagggagctcaaaatggaggacgcggcgctcgggagagcgggcgggtgagtcacccacacaaaggaaaagggcctttccgtcctcagccgtcgcttcatgtgactccacggagtaccgggcgccgtccaggcacctcgattagttctcgagcttttggagtacgtcgtctttaggttggggggaggggttttatgcgatggagtttccccacactgagtgggtggagactgaagttaggccagcttggcacttgatgtaattctccttggaatttgccctttttgagtttggatcttggttcattctcaagcctcagacagtggttcaaagtttttttcttccatttcaggtgtcgtgattcgaattcgccgccaccatggagacagacacactcctgctatgggtgctgctgctctgggttccaggttccacaggtggcgcagaggcgggtatcaccgggacatggtacaaccaacacggaagcacatttacagtcaccgctggagcagacgggaatctgaccggacagtacgagaacagggctcaggggacaggttgtcagaacagtccgtatactctgactgggaggtacaatggcacgaagctggagtggcgagtcgagtggaataattccacggaaaactgtcacagtagaacagagtggaggggacagtaccaggggggagcagaggcccggatcaacacccaatggaacttgacatatgaaggcgggtcaggccccgcgacagagcaaggacaggatacattcacgaaggtcaagccaagcgcagcctctggctctaccacaactccagctccccggccccctactcctgctccaaccattgcctcacagccactgagcctgcggcccgaagcttgtagacctgctgctggaggagctgtgcataccagaggcctggacttcgcctgcgatatgttctgggtgctggtggtggtgggcggggtgctggcctgctacagcctgctggtgacagtggccttcatcatcttttgggtgaaacggggcagaaagaaactcctgtatatattcaaacaaccatttatgagaccagtacaaactactcaagaggaagatggctgtagctgccgatttccagaagaagaagaaggaggatgtgaactgcgggtgaagttcagcagaagcgccgacgcccctgcctaccagcagggccagaatcagctgtacaacgagctgaacctgggcagaagggaagagtacgacgtcctggataagcggagaggccgggaccctgagatgggcggcaagcctcggcggaagaacccccaggaaggcctgtataacgaactgcagaaagacaagatggccgaggcctacagcgagatcggcatgaagggcgagcggaggcggggcaagggccacgacggcctgtatcagggcctgtccaccgccaccaaggatacctacgacgccctgcacatgcaggccctgcccccaagggagggcagaggcagcctgctgacatgtggcgacgtggaagagaaccctggccccatggtgagcaagggcgaggagctgttcaccggggtggtgcccatcctggtcgagctggacggcgacgtaaacggccacaagttcagcgtgtccggcgagggcgagggcgatgccacctacggcaagctgaccctgaagttcatctgcaccaccggcaagctgcccgtgccctggcccaccctcgtgaccaccctgacctacggcgtgcagtgcttcagccgctaccccgaccacatgaagcagcacgacttcttcaagtccgccatgcccgaaggctacgtccaggagcgcaccatcttcttcaaggacgacggcaactacaagacccgcgccgaggtgaagttcgagggcgacaccctggtgaaccgcatcgagctgaagggcatcgacttcaaggaggacggcaacatcctggggcacaagctggagtacaactacaacagccacaacgtctatatcatggccgacaagcagaagaacggcatcaaggtgaacttcaagatccgccacaacatcgaggacggcagcgtgcagctcgccgaccactaccagcagaacacccccatcggcgacggccccgtgctgctgcccgacaaccactacctgagcacccagtccgccctgagcaaagaccccaacgagaagcgcgatcacatggtcctgctggagttcgtgaccgccgccgggatcactctcggcatggacgagctgtacaagtaatctagaccgcgtctggaacaatcaacctctggattacaaaatttgtgaaagattgactggtattcttaactatgttgctccttttacgctatgtggatacgctgctttaatgcctttgtatcatgctattgcttcccgtatggctttcattttctcctccttgtataaatcctggttgctgtctctttatgaggagttgtggcccgttgtcaggcaacgtggcgtggtgtgcactgtgtttgctgacgcaacccccactggttggggcattgccaccacctgtcagctcctttccgggactttcgctttccccctccctattgccacggcggaactcatcgccgcctgccttgcccgctgctggacaggggctcggctgttgggcactgacaattccgtggtgttgtcggggaagctgacgtcctttccatggctgctcgcctgtgttgccacctggattctgcgcgggacgtccttctgctacgtcccttcggccctcaatccagcggaccttccttcccgcggcctgctgccggctctgcggcctcttccgcgtcttcgccttcgccctcagacgagtcggatctccctttgggccgcctccccgcctggaattaattctgcagtcgagacctagaaaaacatggagcaatcacaagtagcaatacagcagctaccaatgctgattgtgcctggctagaagcacaagaggaggaggaggtgggttttccagtcacacctcaggtacctttaagaccaatgacttacaaggcagctgtagatcttagccactttttaaaagaaaagaggggactggaagggctaattcactcccaacgaagacaagatatccttgatctgtggatctaccacacacaaggctacttccctgattagcagaactacacaccagggccaggggtcagatatccactgacctttggatggtgctacaagctagtaccagttgagccagataaggtagaagaggccaataaaggagagaacaccagcttgttacaccctgtgagcctgcatgggatggatgacccggagagagaagtgttagagtggaggtttgacagccgcctagcatttcatcacgtggcccgagagctgcatccggagtacttcaagaactgctgatatcgagcttgctacaagggactttccgctggggactttccagggaggcgtggcctgggcgggactggggagtggcgagccctcagatcctgcatataagcagctgctttttgcctgtactgggtctctctggttagaccagatctgagcctgggagctctctggctaactagggaacccactgcttaagcctcaataaagcttgccttgagtgcttcaagtagtgtgtgcccgtctgttgtgtgactctggtaactagagatccctcagacccttttagtcagtgtggaaaatctctagcagtagtagttcatgtcatcttattattcagtatttataacttgcaaagaaatgaatatcagagagtgagaggccttgacattgctagcgttttaccgtcgacctctagctagagcttggcgtaatcatggtcatagctgtttcctgtgtgaaattgttatccgctcacaattccacacaacatacgagccggaagcataaagtgtaaagcctggggtgcctaatgagtgagctaactcacattaattgcgttgcgctcactgcccgctttccagtcgggaaacctgtcgtgccagctgcattaatgaatcggccaacgcgcggggagaggcggtttgcgtattgggcgctcttccgcttcctcgctcactgactcgctgcgctcggtcgttcggctgcggcgagcggtatcagctcactcaaaggcggtaatacggttatccacagaatcaggggataacgcaggaaagaacatgtgagcaaaaggccagcaaaaggccaggaaccgtaaaaaggccgcgttgctggcgtttttccataggctccgcccccctgacgagcatcacaaaaatcgacgctcaagtcagaggtggcgaaacccgacaggactataaagataccaggcgtttccccctggaagctccctcgtgcgctctcctgttccgaccctgccgcttaccggatacctgtccgcctttctcccttcgggaagcgtggcgctttctcatagctcacgctgtaggtatctcagttcggtgtaggtcgttcgctccaagctgggctgtgtgcacgaaccccccgttcagcccgaccgctgcgccttatccggtaactatcgtcttgagtccaacccggtaagacacgacttatcgccactggcagcagccactggtaacaggattagcagagcgaggtatgtaggcggtgctacagagttcttgaagtggtggcctaactacggctacactagaagaacagtatttggtatctgcgctctgctgaagccagttaccttcggaaaaagagttggtagctcttgatccggcaaacaaaccaccgctggtagcggtggtttttttgtttgcaagcagcagattacgcgcagaaaaaaaggatctcaagaagatcctttgatcttttctacggggtctgacgctcagtggaacgaaaactcacgttaagggattttggtcatgagattatcaaaaaggatcttcacctagatccttttaaattaaaaatgaagttttaaatcaatctaaagtatatatgagtaaacttggtctgacagttaccaatgcttaatcagtgaggcacctatctcagcgatctgtctatttcgttcatccatagttgcctgactccccgtcgtgtagataactacgatacgggagggcttaccatctggccccagtgctgcaatgataccgcgagacccacgctcaccggctccagatttatcagcaataaaccagccagccggaagggccgagcgcagaagtggtcctgcaactttatccgcctccatccagtctattaattgttgccgggaagctagagtaagtagttcgccagttaatagtttgcgcaacgttgttgccattgctacaggcatcgtggtgtcacgctcgtcgtttggtatggcttcattcagctccggttcccaacgatcaaggcgagttacatgatcccccatgttgtgcaaaaaagcggttagctccttcggtcctccgatcgttgtcagaagtaagttggccgcagtgttatcactcatggttatggcagcactgcataattctcttactgtcatgccatccgtaagatgcttttctgtgactggtgagtactcaaccaagtcattctgagaatagtgtatgcggcgaccgagttgctcttgcccggcgtcaatacgggataataccgcgccacatagcagaactttaaaagtgctcatcattggaaaacgttcttcggggcgaaaactctcaaggatcttaccgctgttgagatccagttcgatgtaacccactcgtgcacccaactgatcttcagcatcttttactttcaccagcgtttctgggtgagcaaaaacaggaaggcaaaatgccgcaaaaaagggaataagggcgacacggaaatgttgaatactcatactcttcctttttcaatattattgaagcatttatcagggttattgtctcatgagcggatacatatttgaatgtatttagaaaaataaacaaataggggttccgcgcacatttccccgaaaagtgccacctgacgtcgacggatcgggagatcaacttgtttattgcagcttataatggttacaaataaagcaatagcatcacaaatttcacaaataaagcatttttttcactgcattctagttgtggtttgtccaaactcatcaatgtatcttatcatgtctggatcaactggataactcaagctaaccaaaatcatcccaaacttcccaccccataccctattaccactgccaattacctgtggtttcatttactctaaacctgtgattcctctgaattattttcattttaaagaaattgtatttgttaaatatgtactacaaacttagtagtttttaaagaaattgtatttgttaaatatgtactacaaacttagtagt

SEQ ID NO: 9 - protein, 44 aa, Homo sapiens
  source 1..44: note = CD28 signalling domain
RSKRSRGGHSDYMNMTPRRPGPTRKHYQPYAPPRDFAAYRSGGG

SEQ ID NO: 10 - protein, 371 aa, synthetic construct
  source 1..371: note = CARCD28
METDTLLLWVLLLWVPGSTGGAEAGITGTWYNQHGSTFTVTAGADGNLTGQYENRAQGTGCQNSPYTLTGRYNGTKLEWRVEWNNSTENCHSRTEWRGQYQGGAEARINTQWNLTYEGGSGPATEQGQDTFTKVKPSAASGSTTTPAPRPPTPAPTIASQPLSLRPEACRPAAGGAVHTRGLDFACDMFWVLVVVGGVLACYSLLVTVAFIIFWVRSKRSRGGHSDYMNMTPRRPGPTRKHYQPYAPPRDFAAYRSGGGRVKFSRSADAPAYQQGQNQLYNELNLGRREEYDVLDKRRGRDPEMGGKPRRKNPQEGLYNELQKDKMAEAYSEIGMKGERRRGKGHDGLYQGLSTATKDTYDALHMQALPPR

SEQ ID NO: 11 - DNA, 9523 bp, synthetic construct
  source 1..9523: mol_type = other DNA; note = Expression construct
tggaagggctaattcactcccaaagaagacaagatatccttgatctgtggatctaccacacacaaggctacttccctgattagcagaactacacaccagggccaggggtcagatatccactgacctttggatggtgctacaagctagtaccagttgagccagataaggtagaagaggccaataaaggagagaacaccagcttgttacaccctgtgagcctgcatgggatggatgacccggagagagaagtgttagagtggaggtttgacagccgcctagcatttcatcacgtggcccgagagctgcatccggagtacttcaagaactgctgatatcgagcttgctacaagggactttccgctggggactttccagggaggcgtggcctgggcgggactggggagtggcgagccctcagatcctgcatataagcagctgctttttgcctgtactgggtctctctggttagaccagatctgagcctgggagctctctggctaactagggaacccactgcttaagcctcaataaagcttgccttgagtgcttcaagtagtgtgtgcccgtctgttgtgtgactctggtaactagagatccctcagacccttttagtcagtgtggaaaatctctagcagtggcgcccgaacagggacttgaaagcgaaagggaaaccagaggagctctctcgacgcaggactcggcttgctgaagcgcgcacggcaagaggcgaggggcggcgactggtgagtacgccaaaaattttgactagcggaggctagaaggagagagatgggtgcgagagcgtcagtattaagcgggggagaattagatcgcgatgggaaaaaattcggttaaggccagggggaaagaaaaaatataaattaaaacatatagtatgggcaagcagggagctagaacgattcgcagttaatcctggcctgttagaaacatcagaaggctgtagacaaatactgggacagctacaaccatcccttcagacaggatcagaagaacttagatcattatataatacagtagcaaccctctattgtgtgcatcaaaggatagagataaaagacaccaaggaagctttagacaagatagaggaagagcaaaacaaaagtaagaccaccgcacagcaagcggccggccgctgatcttcagacctggaggaggagatatgagggacaattggagaagtgaattatataaatataaagtagtaaaaattgaaccattaggagtagcacccaccaaggcaaagagaagagtggtgcagagagaaaaaagagcagtgggaataggagctttgttccttgggttcttgggagcagcaggaagcactatgggcgcagcgtcaatgacgctgacggtacaggccagacaattattgtctggtatagtgcagcagcagaacaatttgctgagggctattgaggcgcaacagcatctgttgcaactcacagtctggggcatcaagcagctccaggcaagaatcctggctgtggaaagatacctaaaggatcaacagctcctggggatttggggttgctctggaaaactcatttgcaccactgctgtgccttggaatgctagttggagtaataaatctctggaacagatttggaatcacacgacctggatggagtgggacagagaaattaacaattacacaagcttaatacactccttaattgaagaatcgcaaaaccagcaagaaaagaatgaacaagaattattggaattagataaatgggcaagtttgtggaattggtttaacataacaaattggctgtggtatataaaattattcataatgatagtaggaggcttggtaggtttaagaatagtttttgctgtactttctatagtgaatagagttaggcagggatattcaccattatcgtttcagacccacctcccaaccccgaggggacccgacaggcccgaaggaatagaagaagaaggtggagagagagacagagacagatccattcgattagtgaacggatctcgacggtatcgcctttaaaagaaaaggggggattggggggtacagtgcaggggaaagaatagtagacataatagcaacagacatacaaactaaagaattacaaaaacaaattacaaaaattcaaaattttcgggtttattacagggacagcagagatccagtttatcgatgagtaattcatacaaaaggactcgcccctgccttggggaatcccagggaccgtcgttaaactcccactaacgtagaacccagagatcgctgcgttcccgccccctcacccgcccgctctcgtcatcactgaggtggagaagagcatgcgtgaggctccggtgcccgtcagtgggcagagcgcacatcgcccacagtccccgagaagttggggggaggggtcggcaattgaaccggtgcctagagaaggtggcgcggggtaaactgggaaagtgatgtcgtgtactggctccgcctttttcccgagggtgggggagaaccgtatataagtgcagtagtcgccgtgaacgttctttttcgcaacgggtttgccgccagaacacaggtaagtgccgtgtgtggttcccgcgggcctggcctctttacgggttatggcccttgcgtgccttgaattacttccacgcccctggctgcagtacgtgattcttgatcccgagcttcgggttggaagtgggtgggagagttcgaggccttgcgcttaaggagccccttcgcctcgtgcttgagttgaggcctggcttgggcgctggggccgccgcgtgcgaatctggtggcaccttcgcgcctgtctcgctgctttcgataagtctctagccatttaaaatttttgatgacctgctgcgacgctttttttctggcaagatagtcttgtaaatgcgggccaagatctgcacactggtatttcggtttttggggccgcgggcggcgacggggcccgtgcgtcccagcgcacatgttcggcgaggcggggcctgcgagcgcggccaccgagaatcggacgggggtagtctcaagctggccggcctgctctggtgcctggcctcgcgccgccgtgtatcgccccgccctgggcggcaaggctggcccggtcggcaccagttgcgtgagcggaaagatggccgcttcccggccctgctgcagggagctcaaaatggaggacgcggcgctcgggagagcgggcgggtgagtcacccacacaaaggaaaagggcctttccgtcctcagccgtcgcttcatgtgactccacggagtaccgggcgccgtccaggcacctcgattagttctcgagcttttggagtacgtcgtctttaggttggggggaggggttttatgcgatggagtttccccacactgagtgggtggagactgaagttaggccagcttggcacttgatgtaattctccttggaatttgccctttttgagtttggatcttggttcattctcaagcctcagacagtggttcaaagtttttttcttccatttcaggtgtcgtgattcgaattcgccgccaccatggagacagacacactcctgctatgggtgctgctgctctgggttccaggttccacaggtggcgcagaggcgggtatcaccgggacatggtacaaccaacacggaagcacatttacagtcaccgctggagcagacgggaatctgaccggacagtacgagaacagggctcaggggacaggttgtcagaacagtccgtatactctgactgggaggtacaatggcacgaagctggagtggcgagtcgagtggaataattccacggaaaactgtcacagtagaacagagtggaggggacagtaccaggggggagcagaggcccggatcaacacccaatggaacttgacatatgaaggcgggtcaggccccgcgacagagcaaggacaggatacattcacgaaggtcaagccaagcgcagcctctggctctaccacaactccagctccccggccccctactcctgctccaaccattgcctcacagccactgagcctgcggcccgaagcttgtagacctgctgctggaggagctgtgcataccagaggcctggacttcgcctgcgatatgttctgggtgctggtggtggtgggcggggtgctggcctgctacagcctgctggtgacagtggccttcatcatcttttgggtgcggagcaagcggagcagaggcggccacagcgactacatgaacatgacccccagacggcctggccccacccggaagcactaccagccctacgccccacccagggactttgccgcctaccggtccggcggagggcgggtgaagttcagcagaagcgccgacgcccctgcctaccagcagggccagaatcagctgtacaacgagctgaacctgggcagaagggaagagtacgacgtcctggataagcggagaggccgggaccctgagatgggcggcaagcctcggcggaagaacccccaggaaggcctgtataacgaactgcagaaagacaagatggccgaggcctacagcgagatcggcatgaagggcgagcggaggcggggcaagggccacgacggcctgtatcagggcctgtccaccgccaccaaggatacctacgacgccctgcacatgcaggccctgcccccaagggagggcagaggcagcctgctgacatgtggcgacgtggaagagaaccctggccccatggtgagcaagggcgaggagctgttcaccggggtggtgcccatcctggtcgagctggacggcgacgtaaacggccacaagttcagcgtgtccggcgagggcgagggcgatgccacctacggcaagctgaccctgaagttcatctgcaccaccggcaagctgcccgtgccctggcccaccctcgtgaccaccctgacctacggcgtgcagtgcttcagccgctaccccgaccacatgaagcagcacgacttcttcaagtccgccatgcccgaaggctacgtccaggagcgcaccatcttcttcaaggacgacggcaactacaagacccgcgccgaggtgaagttcgagggcgacaccctggtgaaccgcatcgagctgaagggcatcgacttcaaggaggacggcaacatcctggggcacaagctggagtacaactacaacagccacaacgtctatatcatggccgacaagcagaagaacggcatcaaggtgaacttcaagatccgccacaacatcgaggacggcagcgtgcagctcgccgaccactaccagcagaacacccccatcggcgacggccccgtgctgctgcccgacaaccactacctgagcacccagtccgccctgagcaaagaccccaacgagaagcgcgatcacatggtcctgctggagttcgtgaccgccgccgggatcactctcggcatggacgagctgtacaagtaatctagaccgcgtctggaacaatcaacctctggattacaaaatttgtgaaagattgactggtattcttaactatgttgctccttttacgctatgtggatacgctgctttaatgcctttgtatcatgctattgcttcccgtatggctttcattttctcctccttgtataaatcctggttgctgtctctttatgaggagttgtggcccgttgtcaggcaacgtggcgtggtgtgcactgtgtttgctgacgcaacccccactggttggggcattgccaccacctgtcagctcctttccgggactttcgctttccccctccctattgccacggcggaactcatcgccgcctgccttgcccgctgctggacaggggctcggctgttgggcactgacaattccgtggtgttgtcggggaagctgacgtcctttccatggctgctcgcctgtgttgccacctggattctgcgcgggacgtccttctgctacgtcccttcggccctcaatccagcggaccttccttcccgcggcctgctgccggctctgcggcctcttccgcgtcttcgccttcgccctcagacgagtcggatctccctttgggccgcctccccgcctggaattaattctgcagtcgagacctagaaaaacatggagcaatcacaagtagcaatacagcagctaccaatgctgattgtgcctggctagaagcacaagaggaggaggaggtgggttttccagtcacacctcaggtacctttaagaccaatgacttacaaggcagctgtagatcttagccactttttaaaagaaaagaggggactggaagggctaattcactcccaacgaagacaagatatccttgatctgtggatctaccacacacaaggctacttccctgattagcagaactacacaccagggccaggggtcagatatccactgacctttggatggtgctacaagctagtaccagttgagccagataaggtagaagaggccaataaaggagagaacaccagcttgttacaccctgtgagcctgcatgggatggatgacccggagagagaagtgttagagtggaggtttgacagccgcctagcatttcatcacgtggcccgagagctgcatccggagtacttcaagaactgctgatatcgagcttgctacaagggactttccgctggggactttccagggaggcgtggcctgggcgggactggggagtggcgagccctcagatcctgcatataagcagctgctttttgcctgtactgggtctctctggttagaccagatctgagcctgggagctctctggctaactagggaacccactgcttaagcctcaataaagcttgccttgagtgcttcaagtagtgtgtgcccgtctgttgtgtgactctggtaactagagatccctcagacccttttagtcagtgtggaaaatctctagcagtagtagttcatgtcatcttattattcagtatttataacttgcaaagaaatgaatatcagagagtgagaggccttgacattgctagcgttttaccgtcgacctctagctagagcttggcgtaatcatggtcatagctgtttcctgtgtgaaattgttatccgctcacaattccacacaacatacgagccggaagcataaagtgtaaagcctggggtgcctaatgagtgagctaactcacattaattgcgttgcgctcactgcccgctttccagtcgggaaacctgtcgtgccagctgcattaatgaatcggccaacgcgcggggagaggcggtttgcgtattgggcgctcttccgcttcctcgctcactgactcgctgcgctcggtcgttcggctgcggcgagcggtatcagctcactcaaaggcggtaatacggttatccacagaatcaggggataacgcaggaaagaacatgtgagcaaaaggccagcaaaaggccaggaaccgtaaaaaggccgcgttgctggcgtttttccataggctccgcccccctgacgagcatcacaaaaatcgacgctcaagtcagaggtggcgaaacccgacaggactataaagataccaggcgtttccccctggaagctccctcgtgcgctctcctgttccgaccctgccgcttaccggatacctgtccgcctttctcccttcgggaagcgtggcgctttctcatagctcacgctgtaggtatctcagttcggtgtaggtcgttcgctccaagctgggctgtgtgcacgaaccccccgttcagcccgaccgctgcgccttatccggtaactatcgtcttgagtccaacccggtaagacacgacttatcgccactggcagcagccactggtaacaggattagcagagcgaggtatgtaggcggtgctacagagttcttgaagtggtggcctaactacggctacactagaagaacagtatttggtatctgcgctctgctgaagccagttaccttcggaaaaagagttggtagctcttgatccggcaaacaaaccaccgctggtagcggtggtttttttgtttgcaagcagcagattacgcgcagaaaaaaaggatctcaagaagatcctttgatcttttctacggggtctgacgctcagtggaacgaaaactcacgttaagggattttggtcatgagattatcaaaaaggatcttcacctagatccttttaaattaaaaatgaagttttaaatcaatctaaagtatatatgagtaaacttggtctgacagttaccaatgcttaatcagtgaggcacctatctcagcgatctgtctatttcgttcatccatagttgcctgactccccgtcgtgtagataactacgatacgggagggcttaccatctggccccagtgctgcaatgataccgcgagacccacgctcaccggctccagatttatcagcaataaaccagccagccggaagggccgagcgcagaagtggtcctgcaactttatccgcctccatccagtctattaattgttgccgggaagctagagtaagtagttcgccagttaatagtttgcgcaacgttgttgccattgctacaggcatcgtggtgtcacgctcgtcgtttggtatggcttcattcagctccggttcccaacgatcaaggcgagttacatgatcccccatgttgtgcaaaaaagcggttagctccttcggtcctccgatcgttgtcagaagtaagttggccgcagtgttatcactcatggttatggcagcactgcataattctcttactgtcatgccatccgtaagatgcttttctgtgactggtgagtactcaaccaagtcattctgagaatagtgtatgcggcgaccgagttgctcttgcccggcgtcaatacgggataataccgcgccacatagcagaactttaaaagtgctcatcattggaaaacgttcttcggggcgaaaactctcaaggatcttaccgctgttgagatccagttcgatgtaacccactcgtgcacccaactgatcttcagcatcttttactttcaccagcgtttctgggtgagcaaaaacaggaaggcaaaatgccgcaaaaaagggaataagggcgacacggaaatgttgaatactcatactcttcctttttcaatattattgaagcatttatcagggttattgtctcatgagcggatacatatttgaatgtatttagaaaaataaacaaataggggttccgcgcacatttccccgaaaagtgccacctgacgtcgacggatcgggagatcaacttgtttattgcagcttataatggttacaaataaagcaatagcatcacaaatttcacaaataaagcatttttttcactgcattctagttgtggtttgtccaaactcatcaatgtatcttatcatgtctggatcaactggataactcaagctaaccaaaatcatcccaaacttcccaccccataccctattaccactgccaattacctgtggtttcatttactctaaacctgtgattcctctgaattattttcattttaaagaaattgtatttgttaaatatgtactacaaacttagtagtttttaaagaaattgtatttgttaaatatgtactacaaacttagtagt

SEQ ID NO: 12 - protein, 86 aa, synthetic construct
  source 1..86: note = Fused CD28 and 41-BB sequences
RSKRSRGGHSDYMNMTPRRPGPTRKHYQPYAPPRDFAAYRSGGGKRGRKKLLYIFKQPFMRPVQTTQEEDGCSCRFPEEEEGGCEL